European Patent Application EP 4 223 308 A1, published August 9, 2023. Title: A Composition for preventing or treating Neurological disorders comprising placental growth factor. Applicant: University-Industry Cooperation Group of Kyung Hee University Hankuk University OF Foreign Studies Research and Business Foundation. The sequence listing filed with the application follows.

SEQUENCE LISTING (8 sequences)

SEQ ID NO: 1 - protein, 170 aa, Unknown
  PLGF amino acid (isoform 1)
MPVMRLFPCFLQLLAGLALPAVPPQQWALSAGNGSSEVEVVPFQEVWGRSYCRALERLVDVVSEYPSEVEHMFSPSCVSLLRCTGCCGDENLHCVPVETANVTMQLLKIRSGDRPSYVELTFSQHVRCECRPLREKMKPERRRPKGRGKRRREKQRPTDCHLCGDAVPRR

SEQ ID NO: 2 - protein, 170 aa, Unknown; identical to SEQ ID NO: 1
  PLGF amino acid (isoform 2)

SEQ ID NO: 3 - protein, 221 aa, Unknown
  PLGF amino acid (isoform 3)
MPVMRLFPCFLQLLAGLALPAVPPQQWALSAGNGSSEVEVVPFQEVWGRSYCRALERLVDVVSEYPSEVEHMFSPSCVSLLRCTGCCGDENLHCVPVETANVTMQLLKIRSGDRPSYVELTFSQHVRCECRHSPGRQSPDMPGDFRADAPSFLPPRRSLPMLFRMEWGCALTGSQSAVWPSSPVPEEIPRMHPGRNGKKQQRKPLREKMKPERCGDAVPRR

SEQ ID NO: 4 - DNA, 513 bp, Unknown
  PLGF nucleotide (isoform 1)
atgccggtcatgaggctgttcccttgcttcctgcagctcctggccgggctggcgctgcctgctgtgcccccccagcagtgggccttgtctgctgggaacggctcgtcagaggtggaagtggtacccttccaggaagtgtggggccgcagctactgccgggcgctggagaggctggtggacgtcgtgtccgagtaccccagcgaggtggagcacatgttcagcccatcctgtgtctccctgctgcgctgcaccggctgctgcggcgatgagaatctgcactgtgtgccggtggagacggccaatgtcaccatgcagctcctaaagatccgttctggggaccggccctcctacgtggagctgacgttctctcagcacgttcgctgcgaatgccggcctctgcgggagaagatgaagccggaaaggaggagacccaagggcagggggaagaggaggagagagaagcagagacccacagactgccacctgtgcggcgatgctgttccccggaggtaa

SEQ ID NO: 5 - DNA, 507 bp, Unknown
  PLGF nucleotide (isoform 2)
atgccggtcatgaggctgttcccttgcttcctgcagctcctggccgggctggcgctgcctgctgtgcccccccagcagtgggccttgtctgctgggaacggctcgtcagaggtggaagtggtacccttccaggaagtgtggggccgcagctactgccgggcgctggagaggctggtggacgtcgtgtccgagtaccccagcgaggtggagcacatgttcagcccatcctgtgtctccctgctgcgctgcaccggctgctgcggcgatgagaatctgcactgtgtgccggtgagacggccaatgtcaccatgcagctcctaaagatccgtctggggaccggccctcctacgtggagctgacgttctctcagcacgttcgctgcgaatgccggcctctgcgggagaagatgaagccggaaaggaggagacccaagggcagggggaagaggaggagagagagcagagacccacagactgccacctgtgcggcgatgctgttccccggagg

SEQ ID NO: 6 - DNA, 215 bp, Unknown
  PLGF nucleotide (isoform 3)
ctttctttgctgcttttttccgttccttccagggtgcattctgggaatttcctcagggacaggagatgatggccagacagcggactggctcctgtcagggcacagccccactccatccggaacaacatggggagtgagcgacggggtgggaggaaggagggagcatcagccctgaagtcaccaggcatgtctgggctctgcctcccagggctgtg

SEQ ID NO: 7 - DNA, 6089 bp, Artificial Sequence
  hPLGF- AAV2
agcgcccaatacgcaaaccgcctctccccgcgcgttggccgattcattaatgcagctgcgcgctcgctcgctcactgaggccgcccgggcaaagcccgggcgtcgggcgacctttggtcgcccggcctcagtgagcgagcgagcgcgcagagagggagtggccaactccatcactaggggttccttgtagttaatgattaacccgccatgctacttatctacgtagccatgctctaggaagatcgtaccattgacgtcaataatgacgtatgttcccatagtaacgccaatagggactttccattgacgtcaatgggtggactatttacggtaaactgcccacttggcagtacatcaagtgtatcatatgccaagtacgccccctattgacgtcaatgacggtaaatggcccgcctggcattatgcccagtacatgaccttatgggactttcctacttggcagtacatctacgtattagtcatcgctattaccatggtcgaggtgagccccacgttctgcttcactctccccatctcccccccctccccacccccaattttgtatttatttattttttaattattttgtgcagcgatgggggcggggggggggggggggcgcgcgccaggcggggcggggcggggcgaggggcggggcggggcgaggcggagaggtgcggcggcagccaatcagagcggcgcgctccgaaagtttccttttatggcgaggcggcggcggcggcggccctataaaaagcgaagcgcgcggcgggcgggagtcgctgcgacgctgccttcgccccgtgccccgctccgccgccgcctcgcgccgcccgccccggctctgactgaccgcgttactcccacaggtgagcgggcgggacggcccttctcctccgggctgtaattagcgcttggtttaatgacggcttgtttcttttctgtggctgcgtgaaagccttgaggggctccgggagggccctttgtgcggggggagcggctcggggctgtccgcggggggacggctgccttcgggggggacggggcagggcggggttcggcttctggcgtgtgaccggcggctctagagcctctgctaaccatgttcatgccttcttctttttcctacagctcctgggcaacgtgctggttattgtgctgtctcatcattttggcaaagaattggatcgggatccatgccggtcatgaggctgttcccttgcttcctgcagctcctggccgggctggcgctgcctgctgtgcccccccagcagtgggccttgtctgctgggaacggctcgtcagaggtggaagtggtacccttccaggaagtgtggggccgcagctactgccgggcgctggagaggctggtggacgtcgtgtccgagtaccccagcgaggtggagcacatgttcagcccatcctgtgtctccctgctgcgctgcaccggctgctgcggcgatgagaatctgcactgtgtgccggtggagacggccaatgtcaccatgcagctcctaaagatccgttctggggaccggccctcctacgtggagctgacgttctctcagcacgttcgctgcgaatgccggcctctgcgggagaagatgaagccggaaaggaggagacccaagggcagggggaagaggaggagagagaagcagagacccacagactgccacctgtgcggcgatgctgttccccggaggtaaaccggtcgccaccatggtgagcaagggcgaggagctgttcaccggggtggtgcccatcctggtcgagctggacggcgacgtaaacggccacaagttcagcgtgtccggcgagggcgagggcgatgccacctacggcaagctgaccctgaagttcatctgcaccaccggcaagctgcccgtgccctggcccaccctcgtgaccaccctgacctacggcgtgcagtgcttcagccgctaccccgaccacatgaagcagcacgacttcttcaagtccgccatgcccgaaggctacgtccaggagcgcaccatcttcttcaaggacgacggcaactacaagacccgcgccgaggtgaagttcgagggcgacaccctggtgaaccgcatcgagctgaagggcatcgacttcaaggaggacggcaacatcctggggcacaagctggagtacaactacaacagccacaacgtctatatcatggccgacaagcagaagaacggcatcaaggtgaacttcaagatccgccacaacatcgaggacggcagcgtgcagctcgccgaccactaccagcagaacacccccatcggcgacggccccgtgctgctgcccgacaaccactacctgagcacccagtccgccctgagcaaagaccccaacgagaagcgcgatcacatggtcctgctggagttcgtgaccgccgccgggatcactctcggcatggacgagctgtacaagtaaagcggccgcgactctagaattcgatatcaagcttatcgataatcaacctctggattacaaaatttgtgaaagattgactggtattcttaactatgttgctccttttacgctatgtggatacgctgctttaatgcctttgtatcatgctattgcttcccgtatggctttcattttctcctccttgtataaatcctggttgctgtctctttatgaggagttgtggcccgttgtcaggcaacgtggcgtggtgtgcactgtgtttgctgacgcaacccccactggttggggcattgccaccacctgtcagctcctttccgggactttcgctttccccctccctattgccacggcggaactcatcgccgcctgccttgcccgctgctggacaggggctcggctgttgggcactgacaattccgtggtgttgtcggggaaatcatcgtcctttccttggctgctcgcctgtgttgccacctggattctgcgcgggacgtccttctgctacgtcccttcggccctcaatccagcggaccttccttcccgcggcctgctgccggctctgcggcctcttccgcgtcttcgccttcgccctcagacgagtcggatctccctttgggccgcctccccgcatcgataccgtcgacccgggcggccgcttcgagcagacatgataagatacattgatgagtttggacaaaccacaactagaatgcagtgaaaaaaatgctttatttgtgaaatttgtgatgctattgctttatttgtaaccattataagctgcaataaacaagttaacaacaacaattgcattcattttatgtttcaggttcagggggagatgtgggaggttttttaaagcaagtaaaacctctacaaatgtggtaaaatcgataaggatcttcctagagcatggctacgtagataagtagcatggcgggttaatcattaactacaaggaacccctagtgatggagttggccactccctctctgcgcgctcgctcgctcactgaggccgggcgaccaaaggtcgcccgacgcccgggctttgcccgggcggcctcagtgagcgagcgagcgcgcagccttaattaacctaattcactggccgtcgttttacaacgtcgtgactgggaaaaccctggcgttacccaacttaatcgccttgcagcacatccccctttcgccagctggcgtaatagcgaagaggcccgcaccgatcgcccttcccaacagttgcgcagcctgaatggcgaatgggacgcgccctgtagcggcgcattaagcgcggcgggtgtggtggttacgcgcagcgtgaccgctacacttgccagcgccctagcgcccgctcctttcgctttcttcccttcctttctcgccacgttcgccggctttccccgtcaagctctaaatcgggggctccctttagggttccgatttagtgctttacggcacctcgaccccaaaaaacttgattagggtgatggttcacgtagtgggccatcgccctgatagacggtttttcgccctttgacgttggagtccacgttctttaatagtggactcttgttccaaactggaacaacactcaaccctatctcggtctattcttttgatttataagggattttgccgatttcggcctattggttaaaaaatgagctgatttaacaaaaatttaacgcgaattttaacaaaatattaacgcttacaatttaggtggcacttttcggggaaatgtgcgcggaacccctatttgtttatttttctaaatacattcaaatatgtatccgctcatgagacaataaccctgataaatgcttcaataatattgaaaaaggaagagtatgagtattcaacatttccgtgtcgcccttattcccttttttgcggcattttgccttcctgtttttgctcacccagaaacgctggtgaaagtaaaagatgctgaagatcagttgggtgcacgagtgggttacatcgaactggatctcaacagcggtaagatccttgagagttttcgccccgaagaacgttttccaatgatgagcacttttaaagttctgctatgtggcgcggtattatcccgtattgacgccgggcaagagcaactcggtcgccgcatacactattctcagaatgacttggttgagtactcaccagtcacagaaaagcatcttacggatggcatgacagtaagagaattatgcagtgctgccataaccatgagtgataacactgcggccaacttacttctgacaacgatcggaggaccgaaggagctaaccgcttttttgcacaacatgggggatcatgtaactcgccttgatcgttgggaaccggagctgaatgaagccataccaaacgacgagcgtgacaccacgatgcctgtagcaatggcaacaacgttgcgcaaactattaactggcgaactacttactctagcttcccggcaacaattaatagactggatggaggcggataaagttgcaggaccacttctgcgctcggcccttccggctggctggtttattgctgataaatctggagccggtgagcgtgggtctcgcggtatcattgcagcactggggccagatggtaagccctcccgtatcgtagttatctacacgacggggagtcaggcaactatggatgaacgaaatagacagatcgctgagataggtgcctcactgattaagcattggtaactgtcagaccaagtttactcatatatactttagattgatttaaaacttcatttttaatttaaaaggatctaggtgaagatcctttttgataatctcatgaccaaaatcccttaacgtgagttttcgttccactgagcgtcagaccccgtagaaaagatcaaaggatcttcttgagatcctttttttctgcgcgtaatctgctgcttgcaaacaaaaaaaccaccgctaccagcggtggtttgtttgccggatcaagagctaccaactctttttccgaaggtaactggcttcagcagagcgcagataccaaatactgttcttctagtgtagccgtagttaggccaccacttcaagaactctgtagcaccgcctacatacctcgctctgctaatcctgttaccagtggctgctgccagtggcgataagtcgtgtcttaccgggttggactcaagacgatagttaccggataaggcgcagcggtcgggctgaacggggggttcgtgcacacagcccagcttggagcgaacgacctacaccgaactgagatacctacagcgtgagctatgagaaagcgccacgcttcccgaagggagaaaggcggacaggtatccggtaagcggcagggtcggaacaggagagcgcacgagggagcttccagggggaaacgcctggtatctttatagtcctgtcgggtttcgccacctctgacttgagcgtcgatttttgtgatgctcgtcaggggggcggagcctatggaaaaacgccagcaacgcggcctttttacggttcctggccttttgctggccttttgctcacatgttctttcctgcgttatcccctgattctgtggataaccgtattaccgcctttgagtgagctgataccgctcgccgcagccgaacgaccgagcgcagcgagtcagtgagcgaggaagcggaag

SEQ ID NO: 8 - DNA, 720 bp, Unknown
  GFP nucleotide
ttacttgtacagctcgtccatgccgagagtgatcccggcggcggtcacgaactccagcaggaccatgtgatcgcgcttctcgttggggtctttgctcagggcggactgggtgctcaggtagtggttgtcgggcagcagcacggggccgtcgccgatgggggtgttctgctggtagtggtcggcgagctgcacgctgccgtcctcgatgttgtggcggatcttgaagttcaccttgatgccgttcttctgcttgtcggccatgatatagacgttgtggctgttgtagttgtactccagcttgtgccccaggatgttgccgtcctccttgaagtcgatgcccttcagctcgatgcggttcaccagggtgtcgccctcgaacttcacctcggcgcgggtcttgtagttgccgtcgtccttgaagaagatggtgcgctcctggacgtagccttcgggcatggcggacttgaagaagtcgtgctgcttcatgtggtcggggtagcggctgaagcactgcacgccgtaggtcagggtggtcacgagggtgggccagggcacgggcagcttgccggtggtgcagatgaacttcagggtcagcttgccgtaggtggcatcgccctcgccctcgccggacacgctgaacttgtggccgtttacgtcgccgtccagctcgaccaggatgggcaccaccccggtgaacagctcctcgcccttgctcaccat